European Patent Specification EP 3 778 587 B1, published October 4, 2023. Title: Heterocyclic Compound. Applicant: Kyoto University Takeda Pharmaceutical Company Limited. The sequence listing filed with the application follows.

SEQUENCE LISTING (2 sequences)

SEQ ID NO: 1 - DNA, 720 bp, Artificial Sequence
  Emerald Green Fluorescent Protein (EmGFP)
atggtgagcaagggcgaggagctgttcaccggggtggtgcccatcctggtcgagctggacggcgacgtaaacggccacaagttcagcgtgtccggcgagggcgagggcgatgccacctacggcaagctgaccctgaagttcatctgcaccaccggcaagctgcccgtgccctggcccaccctcgtgaccaccttcacctacggcgtgcagtgcttcgcccgctaccccgaccacatgaagcagcacgacttcttcaagtccgccatgcccgaaggctacgtccaggagcgcaccatcttcttcaaggacgacggcaactacaagacccgcgccgaggtgaagttcgagggcgacaccctggtgaaccgcatcgagctgaagggcatcgacttcaaggaggacggcaacatcctggggcacaagctggagtacaactacaacagccacaaggtctatatcaccgccgacaagcagaagaacggcatcaaggtgaacttcaagacccgccacaacatcgaggacggcagcgtgcagctcgccgaccactaccagcagaacacccccatcggcgacggccccgtgctgctgcccgacaaccactacctgagcacccagtccgccctgagcaaagaccccaacgagaagcgcgatcacatggtcctgctggagttcgtgaccgccgccgggatcactctcggcatggacgagctgtacaagtaa

SEQ ID NO: 2 - DNA, 711 bp, Artificial Sequence
  mCherry
atggtgagcaagggcgaggaggataacatggccatcatcaaggagttcatgcgcttcaaggtgcacatggagggctccgtgaacggccacgagttcgagatcgagggcgagggcgagggccgcccctacgagggcacccagaccgccaagctgaaggtgaccaagggtggccccctgcccttcgcctgggacatcctgtcccctcagttcatgtacggctccaaggcctacgtgaagcaccccgccgacatccccgactacttgaagctgtccttccccgagggcttcaagtgggagcgcgtgatgaacttcgaggacggcggcgtggtgaccgtgacccaggactcctccctgcaggacggcgagttcatctacaaggtgaagctgcgcggcaccaacttcccctccgacggccccgtaatgcagaagaagaccatgggctgggaggcctcctccgagcggatgtaccccgaggacggcgccctgaagggcgagatcaagcagaggctgaagctgaaggacggcggccactacgacgctgaggtcaagaccacctacaaggccaagaagcccgtgcagctgcccggcgcctacaacgtcaacatcaagttggacatcacctcccacaacgaggactacaccatcgtggaacagtacgaacgcgccgagggccgccactccaccggcggcatggacgagctgtacaagtag